European Patent Application EP 4 748 400 A1, published May 27, 2026. Title: Conjugate for antigen delivery and its use. Applicant: LG CHEM, LTD. The sequence listing filed with the application follows.

SEQUENCE LISTING (151 sequences)

SEQ ID NO: 1 - protein, 77 aa, synthetic construct
  REGION 1..77: note = UbR_PRT
MQIFVKTLTGKTITLEVEPSDTIENVKAKIQDKEGIPPDQQRLIFAGKQLEDGRTLSDYNIQKESTLHLVLRLRGGR

SEQ ID NO: 2 - protein, 75 aa, synthetic construct [sequence omitted]

SEQ ID NO: 3 - protein, 30 aa, synthetic construct
  REGION 1..30: note = Lamp_N_term_PRT
MDDQRDLISNNEQLPMLGRRPGAPESKCSR

SEQ ID NO: 4 - protein, 29 aa, synthetic construct
  REGION 1..29: note = Lamp_C_term_PRT
DDQRDLISNNEQLPMLGRRPGAPESKCSR

SEQ ID NO: 5 - protein, 48 aa, synthetic construct
  REGION 1..48: note = mODC_N_term_PRT
MLMKQIQSHGFPPEVEEQDDGTLPMSCAQESGMDRHPAACASARINVM

SEQ ID NO: 6 - protein, 47 aa, synthetic construct
  REGION 1..47: note = mODC_C_term_PRT
LMKQIQSHGFPPEVEEQDDGTLPMSCAQESGMDRHPAACASARINVM

SEQ ID NO: 7 - protein, 30 aa, synthetic construct
  REGION 1..30: note = cmyc_N_term_PRT
MHEETPPTTSSDSEEEQEDEEEIDVVSVEK

SEQ ID NO: 8 - protein, 29 aa, synthetic construct
  REGION 1..29: note = cmyc_C_term_PRT
HEETPPTTSSDSEEEQEDEEEIDVVSVEK

SEQ ID NO: 9 - protein, 54 aa, synthetic construct
  REGION 1..54: note = SORT1_N_term_PRT
MKKYVCGGRFLVHRYSVLQQHAEANGVDGVDALDTASHTNKSGYHDDSDEDLLE

SEQ ID NO: 10 - protein, 53 aa, synthetic construct
  REGION 1..53: note = SORT1_C_term_PRT
KKYVCGGRFLVHRYSVLQQHAEANGVDGVDALDTASHTNKSGYHDDSDEDLLE

SEQ ID NO: 11 - protein, 105 aa, synthetic construct
  REGION 1..105: note = TRXwt_N_term_PRT
MVKQIESKTAFQEALDAAGDKLVVVDFSATWCGPCKMIKPFFHSLSEKYSNVIFLEVDVDDCQDVASECEVKCMPTFQFFKKGQKVGEFSGANKEKLEATINELV

SEQ ID NO: 12 - protein, 104 aa, synthetic construct
  REGION 1..104: note = TRXwt_C_term_PRT
VKQIESKTAFQEALDAAGDKLVVVDFSATWCGPCKMIKPFFHSLSEKYSNVIFLEVDVDDCQDVASECEVKCMPTFQFFKKGQKVGEFSGANKEKLEATINELV

SEQ ID NO: 13 - protein, 40 aa, synthetic construct
  REGION 1..40: note = PSBD_PRT
VIAMPSVRKYAREKGVDIRLVQGTGKGGRVLKEDIDAWLA

SEQ ID NO: 14 - protein, 191 aa, synthetic construct
  REGION 1..191: note = TRX-UbR_PRT
MVKQIESKTAFQEALDAAGDKLVVVDFSATWCGPCKMIKPFFHSLSEKYSNVIFLEVDVDDCQDVASECEVKCMPTFQFFKKGQKVGEFSGANKEKLEATINELVGGSGGGGSGGQIFVKTLTGKTITLEVEPSDTIENVKAKIQDKEGIPPDQQRLIFAGKQLEDGRTLSDYNIQKESTLHLVLRLRGGR

SEQ ID NO: 15 - protein, 144 aa, synthetic construct
  REGION 1..144: note = TRX-Lamp_PRT
MVKQIESKTAFQEALDAAGDKLVVVDFSATWCGPCKMIKPFFHSLSEKYSNVIFLEVDVDDCQDVASECEVKCMPTFQFFKKGQKVGEFSGANKEKLEATINELVGGSGGGGSGGDDQRDLISNNEQLPMLGRRPGAPESKCSR

SEQ ID NO: 16 - protein, 162 aa, synthetic construct
  REGION 1..162: note = TRX-mODC_PRT
MVKQIESKTAFQEALDAAGDKLVVVDFSATWCGPCKMIKPFFHSLSEKYSNVIFLEVDVDDCQDVASECEVKCMPTFQFFKKGQKVGEFSGANKEKLEATINELVGGSGGGGSGGLMKQIQSHGFPPEVEEQDDGTLPMSCAQESGMDRHPAACASARINVM

SEQ ID NO: 17 - protein, 144 aa, synthetic construct
  REGION 1..144: note = TRX-cmyc_PRT
MVKQIESKTAFQEALDAAGDKLVVVDFSATWCGPCKMIKPFFHSLSEKYSNVIFLEVDVDDCQDVASECEVKCMPTFQFFKKGQKVGEFSGANKEKLEATINELVGGSGGGGSGGHEETPPTTSSDSEEEQEDEEEIDVVSVEK

SEQ ID NO: 18 - protein, 168 aa, synthetic construct
  REGION 1..168: note = TRX-SORT1_PRT
MVKQIESKTAFQEALDAAGDKLVVVDFSATWCGPCKMIKPFFHSLSEKYSNVIFLEVDVDDCQDVASECEVKCMPTFQFFKKGQKVGEFSGANKEKLEATINELVGGSGGGGSGGKKYVCGGRFLVHRYSVLQQHAEANGVDGVDALDTASHTNKSGYHDDSDEDLLE

SEQ ID NO: 19 - protein, 76 aa, synthetic construct
  REGION 1..76: note = SORT1 w/ TM_PRT
SVPIILAIVGLMLVTVVAGVLIVKKYVCGGRFLVHRYSVLQQHAEANGVDGVDALDTASHTNKSGYHDDSDEDLLE

SEQ ID NO: 20 - protein, 56 aa, synthetic construct
  REGION 1..56: note = Lamp w/ TM_PRT
MDDQRDLISNNEQLPMLGRRPGAPESKCSRGALYTGFSILVTLLLAGQATTAYFLY

SEQ ID NO: 21 - DNA, 231 bp, synthetic construct
  misc_feature 1..231: note = UbR_gene
  source 1..231: mol_type = other DNA
atgcagatcttcgtgaaaaccctgaccggcaagaccatcacactggaagtggaacccagcgacaccatcgagaacgtgaaggccaagatccaggacaaagagggcatccctcctgaccagcagagactgatcttcgccggcaagcagctggaagatggcagaaccctgagcgactacaacatccagaaagagtctaccctgcacctggtgctgagactgagaggtggaaga

SEQ ID NO: 22 - DNA, 225 bp, synthetic construct
  misc_feature 1..225: note = Ub_gene
  source 1..225: mol_type = other DNA
cagatcttcgtgaaaaccctgaccggcaagaccatcacactggaagtggaacccagcgacaccatcgagaacgtgaaggccaagatccaggacaaagagggcatccctcctgaccagcagagactgatcttcgccggcaagcagctggaagatggcagaaccctgagcgactacaacatccagaaagagtctaccctgcacctggtgctgagactgagaggtgga

SEQ ID NO: 23 - DNA, 90 bp, synthetic construct
  misc_feature 1..90: note = Lamp_N_term_gene
  source 1..90: mol_type = other DNA
atggacgaccagagggacctgatcagcaacaacgagcagctgcccatgctcggcagaaggcctggcgctcctgagagcaaatgtagcaga

SEQ ID NO: 24 - DNA, 87 bp, synthetic construct
  misc_feature 1..87: note = Lamp_C_term_gene
  source 1..87: mol_type = other DNA
gacgaccagagggacctgatcagcaacaacgagcagctgcccatgctcggcagaaggcctggcgctcctgagagcaaatgtagcaga

SEQ ID NO: 25 - DNA, 144 bp, synthetic construct
  misc_feature 1..144: note = mODC_N_term_gene
  source 1..144: mol_type = other DNA
atgctgatgaagcagatccagagccacggcttcccacctgaggtggaagaacaggacgatggcaccctgcctatgagctgtgcccaagagtccggcatggatagacatcctgccgcctgtgccagcgccagaatcaatgttatg

SEQ ID NO: 26 - DNA, 141 bp, synthetic construct
  misc_feature 1..141: note = mODC_C_term_gene
  source 1..141: mol_type = other DNA
ctgatgaagcagatccagagccacggcttcccacctgaggtggaagaacaggacgatggcaccctgcctatgagctgtgcccaagagtccggcatggatagacatcctgccgcctgtgccagcgccagaatcaatgttatg

SEQ ID NO: 27 - DNA, 90 bp, synthetic construct
  misc_feature 1..90: note = cmyc_N_term_gene
  source 1..90: mol_type = other DNA
atgcacgaggaaacccctccaaccacaagcagcgacagcgaggaagaacaagaggacgaggaagagatcgacgtcgtcagcgtggaaaag

SEQ ID NO: 28 - DNA, 87 bp, synthetic construct
  misc_feature 1..87: note = cmyc_C_term_gene
  source 1..87: mol_type = other DNA
cacgaggaaacccctccaaccacaagcagcgacagcgaggaagaacaagaggacgaggaagagatcgacgtcgtcagcgtggaaaag

SEQ ID NO: 29 - DNA, 162 bp, synthetic construct
  misc_feature 1..162: note = SORT1_N_term_gene
  source 1..162: mol_type = other DNA
atgaagaaatacgtgtgcggcggcagattcctggtgcacagatatagcgtcctgcagcagcacgccgaggccaatggtgttgatggtgtcgatgccctggataccgccagccacacaaacaagagcggctaccacgacgacagcgacgaggatctgcttgag

SEQ ID NO: 30 - DNA, 159 bp, synthetic construct
  misc_feature 1..159: note = SORT1_C_term_gene
  source 1..159: mol_type = other DNA
aagaaatacgtgtgcggcggcagattcctggtgcacagatatagcgtcctgcagcagcacgccgaggccaatggtgttgatggtgtcgatgccctggataccgccagccacacaaacaagagcggctaccacgacgacagcgacgaggatctgcttgag

SEQ ID NO: 31 - DNA, 315 bp, synthetic construct
  misc_feature 1..315: note = TRXwt_N_term_gene
  source 1..315: mol_type = other DNA
atggtcaagcagatcgagagcaagaccgccttccaagaggcccttgatgccgctggcgataagctggtggtggtggatttttccgccacttggtgcggcccctgcaagatgatcaagccattcttccacagcctgagcgagaagtacagcaacgtgatcttcctggaagtggacgtggacgactgccaggatgtggcctctgagtgcgaagtgaagtgcatgcccaccttccagttcttcaagaaaggccagaaagtgggcgagttcagcggcgccaacaaagagaagctggaagccaccatcaacgaactagtt

SEQ ID NO: 32 - DNA, 312 bp, synthetic construct
  misc_feature 1..312: note = TRXwt_C_term_gene
  source 1..312: mol_type = other DNA
gtcaagcagatcgagagcaagaccgccttccaagaggcccttgatgccgctggcgataagctggtggtggtggatttttccgccacttggtgcggcccctgcaagatgatcaagccattcttccacagcctgagcgagaagtacagcaacgtgatcttcctggaagtggacgtggacgactgccaggatgtggcctctgagtgcgaagtgaagtgcatgcccaccttccagttcttcaagaaaggccagaaagtgggcgagttcagcggcgccaacaaagagaagctggaagccaccatcaacgaactagtt

SEQ ID NO: 33 - DNA, 120 bp, synthetic construct
  misc_feature 1..120: note = PSBD_gene
  source 1..120: mol_type = other DNA
gtgatcgccatgcctagcgtgcggaagtacgccagagaaaaaggcgtggacatccggctggtgcaaggcactggaaaaggcggcagagtgctgaaagaggacatcgacgcttggctggct

SEQ ID NO: 34 - DNA, 573 bp, synthetic construct
  misc_feature 1..573: note = TRX-UbR_gene
  source 1..573: mol_type = other DNA
atggtcaagcagatcgagagcaagaccgccttccaagaggcccttgatgccgctggcgataagctggtggtggtggatttttccgccacttggtgcggcccctgcaagatgatcaagccattcttccacagcctgagcgagaagtacagcaacgtgatcttcctggaagtggacgtggacgactgccaggatgtggcctctgagtgcgaagtgaagtgcatgcccaccttccagttcttcaagaaaggccagaaagtgggcgagttcagcggcgccaacaaagagaagctggaagccaccatcaacgaactagttggcggatctggcggcggaggaagcggaggacagatcttcgtgaaaaccctgaccggcaagaccatcacactggaagtggaacccagcgacaccatcgagaacgtgaaggccaagatccaggacaaagagggcatccctcctgaccagcagagactgatcttcgccggcaagcagctggaagatggcagaaccctgagcgactacaacatccagaaagagtctaccctgcacctggtgctgagactgagaggtggaaga

SEQ ID NO: 35 - DNA, 432 bp, synthetic construct
  misc_feature 1..432: note = TRX-Lamp_gene
  source 1..432: mol_type = other DNA
atggtcaagcagatcgagagcaagaccgccttccaagaggcccttgatgccgctggcgataagctggtggtggtggatttttccgccacttggtgcggcccctgcaagatgatcaagccattcttccacagcctgagcgagaagtacagcaacgtgatcttcctggaagtggacgtggacgactgccaggatgtggcctctgagtgcgaagtgaagtgcatgcccaccttccagttcttcaagaaaggccagaaagtgggcgagttcagcggcgccaacaaagagaagctggaagccaccatcaacgaactagttggcggatctggcggcggaggaagcggaggagacgaccagagggacctgatcagcaacaacgagcagctgcccatgctcggcagaaggcctggcgctcctgagagcaaatgtagcaga

SEQ ID NO: 36 - DNA, 486 bp, synthetic construct
  misc_feature 1..486: note = TRX-mODC_gene
  source 1..486: mol_type = other DNA
atggtcaagcagatcgagagcaagaccgccttccaagaggcccttgatgccgctggcgataagctggtggtggtggatttttccgccacttggtgcggcccctgcaagatgatcaagccattcttccacagcctgagcgagaagtacagcaacgtgatcttcctggaagtggacgtggacgactgccaggatgtggcctctgagtgcgaagtgaagtgcatgcccaccttccagttcttcaagaaaggccagaaagtgggcgagttcagcggcgccaacaaagagaagctggaagccaccatcaacgaactagttggcggatctggcggcggaggaagcggaggactgatgaagcagatccagagccacggcttcccacctgaggtggaagaacaggacgatggcaccctgcctatgagctgtgcccaagagtccggcatggatagacatcctgccgcctgtgccagcgccagaatcaatgttatg

SEQ ID NO: 37 - DNA, 432 bp, synthetic construct
  misc_feature 1..432: note = TRX-cmyc_gene
  source 1..432: mol_type = other DNA
atggtcaagcagatcgagagcaagaccgccttccaagaggcccttgatgccgctggcgataagctggtggtggtggatttttccgccacttggtgcggcccctgcaagatgatcaagccattcttccacagcctgagcgagaagtacagcaacgtgatcttcctggaagtggacgtggacgactgccaggatgtggcctctgagtgcgaagtgaagtgcatgcccaccttccagttcttcaagaaaggccagaaagtgggcgagttcagcggcgccaacaaagagaagctggaagccaccatcaacgaactagttggcggatctggcggcggaggaagcggaggacacgaggaaacccctccaaccacaagcagcgacagcgaggaagaacaagaggacgaggaagagatcgacgtcgtcagcgtggaaaag

SEQ ID NO: 38 - DNA, 504 bp, synthetic construct
  misc_feature 1..504: note = TRX-SORT1_gene
  source 1..504: mol_type = other DNA
atggtgaagcagatcgagagcaagaccgccttccaagaggcccttgatgccgctggcgataagctggtggtggtggatttttccgccacttggtgcggcccctgcaagatgatcaagccattcttccacagcctgagcgagaagtacagcaacgtgatcttcctggaagtggacgtggacgactgccaggatgtggcctctgagtgcgaagtgaagtgcatgcccaccttccagttcttcaagaaaggccagaaagtgggcgagttcagcggcgccaacaaagagaagctggaagccaccatcaacgaactagttggcggatctggcggcggaggaagcggaggaaagaaatacgtgtgcggcggcagattcctggtgcacagatatagcgtcctgcagcagcacgccgaggccaatggtgttgatggtgtcgatgccctggataccgccagccacacaaacaagagcggctaccacgacgacagcgacgaggatctgcttgag

SEQ ID NO: 39 - DNA, 228 bp, synthetic construct
  misc_feature 1..228: note = SORT1 w/ TM_gene
  source 1..228: mol_type = other DNA
agcgtgccaatcatcctggccatcgtgggcctgatgctggttacagtggttgccggcgtgctgatcgttaagaaatacgtgtgcggcggcagattcctggtgcacagatatagcgtcctgcagcagcacgccgaggccaatggtgttgatggtgtcgatgccctggataccgccagccacacaaacaagagcggctaccacgacgacagcgacgaggatctgcttgag

SEQ ID NO: 40 - DNA, 168 bp, synthetic construct
  misc_feature 1..168: note = Lamp w/ TM_gene
  source 1..168: mol_type = other DNA
atggacgaccagagggacctgatcagcaacaacgagcagctgcccatgctcggcagaaggcctggcgctcctgagagcaaatgtagcagaggcgctctgtacaccggctttagcatcctggtcacactgttgctggccggacaggctaccacagcctactttctgtac

SEQ ID NO: 41 - DNA, 202 bp, synthetic construct
  misc_feature 1..202: note = 5UTR_TE
  source 1..202: mol_type = other DNA
ccggcgggtttctgacatccggcgggtttctgacatccggcgggtttctgacatccggcgggtttctgacatccggcgggtttctgacatccggcgggtttctgacatccggcgggtttctgacatccggcgggtttctgacatccggcgggtttctgacatccggcgggtttctgacattcacaaccaggcctccacaacc

SEQ ID NO: 42 - DNA, 278 bp, synthetic construct
  misc_feature 1..278: note = 3UTR_2X_HBB
  source 1..278: mol_type = other DNA
agctcgctttcttgctgtccaatttctattaaaggttcctttgttccctaagtccaactactaaactgggggatattatgaagggccttgagcatctggattctgcctaataaaaaacatttattttcattgctgcggatctagctcgctttcttgctgtccaatttctattaaaggttcctttgttccctaagtccaactactaaactgggggatattatgaagggccttgagcatctggattctgcctaataaaaaacatttattttcattgctgc

SEQ ID NO: 43 - DNA, 30 bp, synthetic construct
  misc_feature 1..30: note = oCCP12G-F1
  source 1..30: mol_type = other DNA
ggaggaagcggaggacagatcttcgtgaaa

SEQ ID NO: 44 - DNA, 25 bp, synthetic construct
  misc_feature 1..25: note = oCCPxxG-R1
  source 1..25: mol_type = other DNA
gcaagaaagcgagctctcgagttta

SEQ ID NO: 45 - DNA, 45 bp, synthetic construct
  misc_feature 1..45: note = oGS-EGFP-F
  source 1..45: mol_type = other DNA
ggcggatctggcggcggaggaagcggaggagtgagcaagggcgag

SEQ ID NO: 46 - DNA, 25 bp, synthetic construct
  misc_feature 1..25: note = oCCPxxG-R1
  source 1..25: mol_type = other DNA
gcaagaaagcgagctctcgagttta

SEQ ID NO: 47 - DNA, 17 bp, synthetic construct
  misc_feature 1..17: note = oM13F
  source 1..17: mol_type = other DNA
gtaaaacgacggccagt

SEQ ID NO: 48 - DNA, 45 bp, synthetic construct
  misc_feature 1..45: note = oGS-EGFP-R
  source 1..45: mol_type = other DNA
tcctccgcttcctccgccgccagatccgcccttgtacagctcgtc

SEQ ID NO: 49 - DNA, 45 bp, synthetic construct
  misc_feature 1..45: note = oCTRXwt-F1
  source 1..45: mol_type = other DNA
ggcggatctggcggcggaggaagcggaggagtcaagcagatcgag

SEQ ID NO: 50 - DNA, 40 bp, synthetic construct
  misc_feature 1..40: note = oCTRXwt-R1
  source 1..40: mol_type = other DNA
gcaagaaagcgagctctcgagtttaaactagttcgttgat

SEQ ID NO: 51 - protein, 27 aa, synthetic construct
  REGION 1..27: note = M44_PRT
EFKHIKAFDRTFANNPGPMVVFATPGM

SEQ ID NO: 52 - DNA, 81 bp, synthetic construct
  misc_feature 1..81: note = M44_GENE
  source 1..81: mol_type = other DNA
gagttcaagcacatcaaggccttcgaccggaccttcgccaacaatcccggacctatggtggtgttcgccacacctggaatg

SEQ ID NO: 53 - protein, 27 aa, synthetic construct
  REGION 1..27: note = M30_PRT
PSKPSFQEFVDWENVSPELNSTDQPFL

SEQ ID NO: 54 - DNA, 81 bp, synthetic construct
  misc_feature 1..81: note = M30_GENE
  source 1..81: mol_type = other DNA
cctagcaagcctagcttccaagagttcgtggactgggagaacgtgtcccctgagctgaactctaccgaccagccatttctc

SEQ ID NO: 55 - protein, 27 aa, synthetic construct
  REGION 1..27: note = M21_PRT
SSPDEVALVEGVQSLGFTYLRLKDNYM

SEQ ID NO: 56 - DNA, 81 bp, synthetic construct
  misc_feature 1..81: note = M21_GENE
  source 1..81: mol_type = other DNA
tcttctccagatgaggtggcactggtggaaggcgtgcagtctctgggcttcacctacctgagactgaaggacaactacatg

SEQ ID NO: 57 - protein, 27 aa, synthetic construct
  REGION 1..27: note = M12_PRT
TPPPEEAMPFEFNGPAQGDHSQPPLQV

SEQ ID NO: 58 - DNA, 81 bp, synthetic construct
  misc_feature 1..81: note = M12_GENE
  source 1..81: mol_type = other DNA
acacctccacctgaagaggccatgcctttcgagttcaacggacccgctcagggcgatcactctcagcctccacttcaagtt

SEQ ID NO: 59 - protein, 27 aa, synthetic construct
  REGION 1..27: note = mTrp2_PRT
PNGTQPQIANCSVYDFFVWLHYYSVRD

SEQ ID NO: 60 - DNA, 81 bp, synthetic construct
  misc_feature 1..81: note = mTrp2_GENE
  source 1..81: mol_type = other DNA
cctaatggaacacagccccagatcgccaactgcagcgtgtacgacttcttcgtgtggctgcactactacagcgtcagagat

SEQ ID NO: 61 - protein, 195 aa, synthetic construct
  REGION 1..195: note = 5 Epitopes_PRT
GGSGGGGSGGEFKHIKAFDRTFANNPGPMVVFATPGMGGSGGGGSGGPSKPSFQEFVDWENVSPELNSTDQPFLGGSGGGGSGGSSPDEVALVEGVQSLGFTYLRLKDNYMGGSGGGGSGGTPPPEEAMPFEFNGPAQGDHSQPPLQVGGSGGGGSGGPNGTQPQIANCSVYDFFVWLHYYSVRDGGSGGGGSGG

SEQ ID NO: 62 - DNA, 585 bp, synthetic construct
  misc_feature 1..585: note = 5 Epitopes_GENE
  source 1..585: mol_type = other DNA
ggcggatctggcggcggaggaagcggaggtgagttcaagcacatcaaggccttcgaccggaccttcgccaacaatcccggacctatggtggtgttcgccacacctggaatgggtggaagcggaggaggcggctctggaggccctagcaagcctagcttccaagagttcgtggactgggagaacgtgtcccctgagctgaactctaccgaccagccatttctcggcggatcaggaggcgggggctccggagggtcttctccagatgaggtggcactggtggaaggcgtgcagtctctgggcttcacctacctgagactgaaggacaactacatgggaggatccggcggcggcggaagcggggggacacctccacctgaagaggccatgcctttcgagttcaacggacccgctcagggcgatcactctcagcctccacttcaagttggcggatctggcggcggcggatcaggtggccctaatggaacacagccccagatcgccaactgcagcgtgtacgacttcttcgtgtggctgcactactacagcgtcagagatggcggcagtggcggaggcggctcaggcgga

SEQ ID NO: 63 - protein, 19 aa, synthetic construct
  REGION 1..19: note = P2A_PRT
ATNFSLLKQAGDVEENPGP

SEQ ID NO: 64 - DNA, 57 bp, synthetic construct
  misc_feature 1..57: note = P2A_GENE
  source 1..57: mol_type = other DNA
gctactaacttcagcctgctgaagcaggctggcgacgtggaggagaaccctggacct

SEQ ID NO: 65 - protein, 238 aa, synthetic construct
  REGION 1..238: note = EGFP_PRT
VSKGEELFTGVVPILVELDGDVNGHKFSVSGEGEGDATYGKLTLKFICTTGKLPVPWPTLVTTLTYGVQCFSRYPDHMKQHDFFKSAMPEGYVQERTIFFKDDGNYKTRAEVKFEGDTLVNRIELKGIDFKEDGNILGHKLEYNYNSHNVYIMADKQKNGIKVNFKIRHNIEDGSVQLADHYQQNTPIGDGPVLLPDNHYLSTQSALSKDPNEKRDHMVLLEFVTAAGITLGMDELYK

SEQ ID NO: 66 - DNA, 717 bp, synthetic construct
  misc_feature 1..717: note = EGFP_GENE
  source 1..717: mol_type = other DNA
gtgagcaagggcgaggagctgttcaccggggtggtgcccatcctggtcgagctggacggcgacgtaaacggccacaagttcagcgtgtccggcgagggcgagggcgatgccacctacggcaagctgaccctgaagttcatctgcaccaccggcaagctgcccgtgccctggcccaccctcgtgaccaccctgacctacggcgtgcagtgcttcagccgctaccccgaccacatgaagcagcacgacttcttcaagtccgccatgcccgaaggctacgtccaggagcgcaccatcttcttcaaggacgacggcaactacaagacccgcgccgaggtgaagttcgagggcgacaccctggtgaaccgcatcgagctgaagggcatcgacttcaaggaggacggcaacatcctggggcacaagctggagtacaactacaacagccacaacgtctatatcatggccgacaagcagaagaacggcatcaaggtgaacttcaagatccgccacaacatcgaggacggcagcgtgcagctcgccgaccactaccagcagaacacccccatcggcgacggccccgtgctgctgcccgacaaccactacctgagcacccagtccgccctgagcaaagaccccaacgagaagcgcgatcacatggtcctgctggagttcgtgaccgccgccgggatcactctcggcatggacgagctgtacaagtaa

SEQ ID NO: 67 - DNA, 90 bp, synthetic construct
  misc_feature 1..90: note = oNUbR-A1-F1
  source 1..90: mol_type = other DNA
caggcctccacaaccggcgcgccaccatgcagatcttcgtgaaaaccctgaccggcaagaccatcacactggaagtggaacccagcgaca

SEQ ID NO: 68 - DNA, 89 bp, synthetic construct
  misc_feature 1..89: note = oUbR-R2
  source 1..89: mol_type = other DNA
cggcgaagatcagtctctgctggtcaggagggatgccctctttgtcctggatcttggccttcacgttctcgatggtgtcgctgggttcc

SEQ ID NO: 69 - DNA, 90 bp, synthetic construct
  misc_feature 1..90: note = oUbR-F3
  source 1..90: mol_type = other DNA
gagactgatcttcgccggcaagcagctggaagatggcagaaccctgagcgactacaacatccagaaagagtctaccctgcacctggtgct

SEQ ID NO: 70 - DNA, 67 bp, synthetic construct
  misc_feature 1..67: note = oNUbR-BE1-R5
  source 1..67: mol_type = other DNA
tccaccagatcctccgcctccggaaccgcctcttccacctctcagtctcagcaccaggtgcagggta

SEQ ID NO: 71 - DNA, 48 bp, synthetic construct
  misc_feature 1..48: note = oCUb-BE1-F1
  source 1..48: mol_type = other DNA
ggcggttccggaggcggaggatctggtggacagatcttcgtgaaaacc

SEQ ID NO: 72 - DNA, 40 bp, synthetic construct
  misc_feature 1..40: note = oCUb-X1-R2
  source 1..40: mol_type = other DNA
gcaagaaagcgagctctcgagtttatccacctctcagtct

SEQ ID NO: 73 - DNA, 68 bp, synthetic construct
  misc_feature 1..68: note = oCmODC-BE1-F1
  source 1..68: mol_type = other DNA
ggcggttccggaggcggaggatctggtggactgatgaagcagatccagagccacggcttcccacctga

SEQ ID NO: 74 - DNA, 70 bp, synthetic construct
  misc_feature 1..70: note = omODC-R2
  source 1..70: mol_type = other DNA
ccggactcttgggcacagctcataggcagggtgccatcgtcctgttcttccacctcaggtgggaagccgt

SEQ ID NO: 75 - DNA, 66 bp, synthetic construct
  misc_feature 1..66: note = omODC-F3
  source 1..66: mol_type = other DNA
tgcccaagagtccggcatggatagacatcctgccgcctgtgccagcgccagaatcaatgttatgta

SEQ ID NO: 76 - DNA, 67 bp, synthetic construct
  misc_feature 1..67: note = oCmODC-X1-R4
  source 1..67: mol_type = other DNA
gcaagaaagcgagctctcgagtttacataacattgattctggcgctggcacaggcggcaggatgtct

SEQ ID NO: 77 - DNA, 41 bp, synthetic construct
  misc_feature 1..41: note = oNmODC-A1-F1
  source 1..41: mol_type = other DNA
caggcctccacaaccggcgcgccaccatgctgatgaagcag

SEQ ID NO: 78 - DNA, 45 bp, synthetic construct
  misc_feature 1..45: note = oNmODC-BE1-R2
  source 1..45: mol_type = other DNA
tccaccagatcctccgcctccggaaccgcccataacattgattct

SEQ ID NO: 79 - DNA, 44 bp, synthetic construct
  misc_feature 1..44: note = oNcmyc-A1-F1
  source 1..44: mol_type = other DNA
caggcctccacaaccggcgcgccaccatgcacgaggaaacccct

SEQ ID NO: 80 - DNA, 45 bp, synthetic construct
  misc_feature 1..45: note = oNcmyc-BE1-R2
  source 1..45: mol_type = other DNA
tccaccagatcctccgcctccggaaccgcccttttccacgctgac

SEQ ID NO: 81 - DNA, 77 bp, synthetic construct
  misc_feature 1..77: note = oCcmyc-BE1-F1
  source 1..77: mol_type = other DNA
ggcggttccggaggcggaggatctggtggacacgaggaaacccctccaaccacaagcagcgacagcgaggaagaaca

SEQ ID NO: 82 - DNA, 87 bp, synthetic construct
  misc_feature 1..87: note = oCcmyc-X1-R2
  source 1..87: mol_type = other DNA
gcaagaaagcgagctctcgagtttacttttccacgctgacgacgtcgatctcttcctcgtcctcttgttcttcctcgctgtcgctgc

SEQ ID NO: 83 - DNA, 85 bp, synthetic construct
  misc_feature 1..85: note = oNIi-A1-F1
  source 1..85: mol_type = other DNA
caggcctccacaaccggcgcgccaccatggacgaccagagggacctgatcagcaacaacgagcagctgcccatgctcggcagaag

SEQ ID NO: 84 - DNA, 78 bp, synthetic construct
  misc_feature 1..78: note = oNIi-BE1-R2
  source 1..78: mol_type = other DNA
tccaccagatcctccgcctccggaaccgcctctgctacatttgctctcaggagcgccaggccttctgccgagcatggg

SEQ ID NO: 85 - DNA, 45 bp, synthetic construct
  misc_feature 1..45: note = oCIi-BE1-F1
  source 1..45: mol_type = other DNA
ggcggttccggaggcggaggatctggtggagacgaccagagggac

SEQ ID NO: 86 - DNA, 40 bp, synthetic construct
  misc_feature 1..40: note = oCIi-X1-R2
  source 1..40: mol_type = other DNA
gcaagaaagcgagctctcgagtttatctgctacatttgct

SEQ ID NO: 87 - DNA, 72 bp, synthetic construct
  misc_feature 1..72: note = oLAMPwTM-1F
  source 1..72: mol_type = other DNA
caggcctccacaaccggcgcgccaccatggacgaccagagggacctgatcagcaacaacgagcagctgccca

SEQ ID NO: 88 - DNA, 39 bp, synthetic construct
  misc_feature 1..39: note = oLAMPwTM-2R
  source 1..39: mol_type = other DNA
agcgccaggccttctgccgagcatgggcagctgctcgtt

SEQ ID NO: 89 - DNA, 71 bp, synthetic construct
  misc_feature 1..71: note = oLAMPwTM-3F
  source 1..71: mol_type = other DNA
aggcctggcgctcctgagagcaaatgtagcagaggcgctctgtacaccggctttagcatcctggtcacact

SEQ ID NO: 90 - DNA, 89 bp, synthetic construct
  misc_feature 1..89: note = oLAMPwTM-4R
  source 1..89: mol_type = other DNA
tccaccagatcctccgcctccggaaccgccgtacagaaagtaggctgtggtagcctgtccggccagcagcagtgtgaccaggatgctaa

SEQ ID NO: 91 - DNA, 56 bp, synthetic construct
  misc_feature 1..56: note = oCSORT-BE1-F1
  source 1..56: mol_type = other DNA
ggcggttccggaggcggaggatctggtggaaagaaatacgtgtgcggcggcagatt

SEQ ID NO: 92 - DNA, 83 bp, synthetic construct
  misc_feature 1..83: note = oSORT-R2
  source 1..83: mol_type = other DNA
agggcatcgacaccatcaacaccattggcctcggcgtgctgctgcaggacgctatatctgtgcaccaggaatctgccgccgca

SEQ ID NO: 93 - DNA, 82 bp, synthetic construct
  misc_feature 1..82: note = oSORT-F3
  source 1..82: mol_type = other DNA
tggtgtcgatgccctggataccgccagccacacaaacaagagcggctaccacgacgacagcgacgaggatctgcttgagtaa

SEQ ID NO: 94 - DNA, 59 bp, synthetic construct
  misc_feature 1..59: note = oCSORT-X1-R4
  source 1..59: mol_type = other DNA
gcaagaaagcgagctctcgagtttactcaagcagatcctcgtcgctgtcgtcgtggtag

SEQ ID NO: 95 - DNA, 44 bp, synthetic construct
  misc_feature 1..44: note = oNSORT-A1-F1
  source 1..44: mol_type = other DNA
caggcctccacaaccggcgcgccaccatgaagaaatacgtgtgc

SEQ ID NO: 96 - DNA, 45 bp, synthetic construct
  misc_feature 1..45: note = oNSORT-BE1-R2
  source 1..45: mol_type = other DNA
tccaccagatcctccgcctccggaaccgccctcaagcagatcctc

SEQ ID NO: 97 - DNA, 75 bp, synthetic construct
  misc_feature 1..75: note = oSORTwTM-1F
  source 1..75: mol_type = other DNA
ggcggttccggaggcggaggatctggtggaagcgtgccaatcatcctggccatcgtgggcctgatgctggttaca

SEQ ID NO: 98 - DNA, 90 bp, synthetic construct
  misc_feature 1..90: note = oSORTwTM-2R
  source 1..90: mol_type = other DNA
cgctatatctgtgcaccaggaatctgccgccgcacacgtatttcttaacgatcagcacgccggcaaccactgtaaccagcatcaggccca

SEQ ID NO: 99 - DNA, 89 bp, synthetic construct
  misc_feature 1..89: note = oSORTwTM-3F
  source 1..89: mol_type = other DNA
ctggtgcacagatatagcgtcctgcagcagcacgccgaggccaatggtgttgatggtgtcgatgccctggataccgccagccacacaaa

SEQ ID NO: 100 - DNA, 87 bp, synthetic construct
  misc_feature 1..87: note = oSORTwTM-4R
  source 1..87: mol_type = other DNA
gcaagaaagcgagctctcgagtttactcaagcagatcctcgtcgctgtcgtcgtggtagccgctcttgtttgtgtggctggcggtat

SEQ ID NO: 101 - DNA, 44 bp, synthetic construct
  misc_feature 1..44: note = oNhTRX-A1-F
  source 1..44: mol_type = other DNA
caggcctccacaaccggcgcgccaccatggtgaagcagatcgag

SEQ ID NO: 102 - DNA, 45 bp, synthetic construct
  misc_feature 1..45: note = oNhTRX-BE1-R
  source 1..45: mol_type = other DNA
tccaccagatcctccgcctccggaaccgcccaccagctcgttgat

SEQ ID NO: 103 - DNA, 87 bp, synthetic construct
  misc_feature 1..87: note = oTRXwt-1F
  source 1..87: mol_type = other DNA
caggcctccacaaccggcgcgccaccatggtcaagcagatcgagagcaagaccgccttccaagaggcccttgatgccgctggcgata

SEQ ID NO: 104 - DNA, 60 bp, synthetic construct
  misc_feature 1..60: note = oTRXwt-2R
  source 1..60: mol_type = other DNA
gcaggggccgcaccaagtggcggaaaaatccaccaccaccagcttatcgccagcggcatc

SEQ ID NO: 105 - DNA, 52 bp, synthetic construct
  misc_feature 1..52: note = oTRXwt-3F
  source 1..52: mol_type = other DNA
gcggcccctgcaagatgatcaagccattcttccacagcctgagcgagaagta

SEQ ID NO: 106 - DNA, 89 bp, synthetic construct
  misc_feature 1..89: note = oTRXwt-4R
  source 1..89: mol_type = other DNA
cgcactcagaggccacatcctggcagtcgtccacgtccacttccaggaagatcacgttgctgtacttctcgctcaggctgtggaagaat

SEQ ID NO: 107 - DNA, 89 bp, synthetic construct
  misc_feature 1..89: note = oTRXwt-5F
  source 1..89: mol_type = other DNA
tggcctctgagtgcgaagtgaagtgcatgcccaccttccagttcttcaagaaaggccagaaagtgggcgagttcagcggcgccaacaaa

SEQ ID NO: 108 - DNA, 81 bp, synthetic construct
  misc_feature 1..81: note = oTRXwt-6R
  source 1..81: mol_type = other DNA
tcctccgcttcctccgccgccagatccgccaactagttcgttgatggtggcttccagcttctctttgttggcgccgctgaa

SEQ ID NO: 109 - DNA, 60 bp, synthetic construct
  misc_feature 1..60: note = oTRXwt-3F1
  source 1..60: mol_type = other DNA
cacttggtgcggcccctgcaagatgatcaagccattcttccacagcctgagcgagaagta

SEQ ID NO: 110 - DNA, 45 bp, synthetic construct
  misc_feature 1..45: note = oChPSBD-BE1-F
  source 1..45: mol_type = other DNA
ggcggttccggaggcggaggatctggtggagtgatcgccatgcct

SEQ ID NO: 111 - DNA, 40 bp, synthetic construct
  misc_feature 1..40: note = oChPSBD-X1-R
  source 1..40: mol_type = other DNA
gcaagaaagcgagctctcgagtttaagccagccaagcgtc

SEQ ID NO: 112 - DNA, 45 bp, synthetic construct
  misc_feature 1..45: note = oEGFP-BE1-F
  source 1..45: mol_type = other DNA
ggcggttccggaggcggaggatctggtggagtgagcaagggcgag

SEQ ID NO: 113 - DNA, 45 bp, synthetic construct
  misc_feature 1..45: note = oEGFP-BE1-R
  source 1..45: mol_type = other DNA
tccaccagatcctccgcctccggaaccgcccttgtacagctcgtc

SEQ ID NO: 114 - DNA, 47 bp, synthetic construct
  misc_feature 1..47: note = Epitope_2_F
  source 1..47: mol_type = other DNA
ggctaccgtctcaaggaagcggaggtgagttcaagcacatcaaggcc

SEQ ID NO: 115 - DNA, 43 bp, synthetic construct
  misc_feature 1..43: note = Epitope_2_R
  source 1..43: mol_type = other DNA
ggctaccgtctctactgccgccatctctgacgctgtagtagtg

SEQ ID NO: 116 - DNA, 86 bp, synthetic construct
  misc_feature 1..86: note = GFP_4_F
  source 1..86: mol_type = other DNA
ggctaccgtctcactactaacttcagcctgctgaagcaggctggcgacgtggaggagaaccctggacctgtgagcaagggcgagga

SEQ ID NO: 117 - DNA, 40 bp, synthetic construct
  misc_feature 1..40: note = GFP_4_R
  source 1..40: mol_type = other DNA
ggctaccgtctctcgagtttacttgtacagctcgtccatg

SEQ ID NO: 118 - DNA, 32 bp, synthetic construct
  misc_feature 1..32: note = cMyc_1_F
  source 1..32: mol_type = other DNA
ggctaccgtctcaccatgcacgaggaaacccc

SEQ ID NO: 119 - DNA, 52 bp, synthetic construct
  misc_feature 1..52: note = cMyc_1_R
  source 1..52: mol_type = other DNA
ggctaccgtctcatcctccgccgccagatccgcccttttccacgctgacgac

SEQ ID NO: 120 - DNA, 33 bp, synthetic construct
  misc_feature 1..33: note = Lamp_1_F
  source 1..33: mol_type = other DNA
ggctaccgtctcaccatggacgaccagagggac

SEQ ID NO: 121 - DNA, 57 bp, synthetic construct
  misc_feature 1..57: note = Lamp_1_R
  source 1..57: mol_type = other DNA
ggctaccgtctcatcctccgccgccagatccgcctctgctacatttgctctcaggag

SEQ ID NO: 122 - DNA, 55 bp, synthetic construct
  misc_feature 1..55: note = Lamp_3_F
  source 1..55: mol_type = other DNA
ggctaccgtctctcagtggcggaggcggctcaggcggagacgaccagagggacct

SEQ ID NO: 123 - DNA, 89 bp, synthetic construct
  misc_feature 1..89: note = Lamp_3_R
  source 1..89: mol_type = other DNA
ggctaccgtctctgtagctccgcttccagcgtaatctggaacatcgtatgggtatccggagccgcctctgctacatttgctctcaggag

SEQ ID NO: 124 - DNA, 55 bp, synthetic construct
  misc_feature 1..55: note = Lamp_TM_1_R
  source 1..55: mol_type = other DNA
ggctaccgtctcatcctccgccgccagatccgccgtacagaaagtaggctgtggt

SEQ ID NO: 125 - DNA, 33 bp, synthetic construct
  misc_feature 1..33: note = mODC_1_F
  source 1..33: mol_type = other DNA
ggctaccgtctcaccatgctgatgaagcagatc

SEQ ID NO: 126 - DNA, 55 bp, synthetic construct
  misc_feature 1..55: note = mODC_1_R
  source 1..55: mol_type = other DNA
ggctaccgtctcatcctccgccgccagatccgcccataacattgattctggcgct

SEQ ID NO: 127 - DNA, 60 bp, synthetic construct
  misc_feature 1..60: note = mODC_3_F
  source 1..60: mol_type = other DNA
ggctaccgtctctcagtggcggaggcggctcaggcggactgatgaagcagatccagagcc

SEQ ID NO: 128 - DNA, 88 bp, synthetic construct
  misc_feature 1..88: note = mODC_3_R
  source 1..88: mol_type = other DNA
ggctaccgtctctgtagctccgcttccagcgtaatctggaacatcgtatgggtatccggagccgcccataacattgattctggcgctg

SEQ ID NO: 129 - DNA, 36 bp, synthetic construct
  misc_feature 1..36: note = SORT1_1_F
  source 1..36: mol_type = other DNA
ggctaccgtctcaccatgaagaaatacgtgtgcggc

SEQ ID NO: 130 - DNA, 53 bp, synthetic construct
  misc_feature 1..53: note = SORT1_1_R
  source 1..53: mol_type = other DNA
ggctaccgtctcatcctccgccgccagatccgccctcaagcagatcctcgtcg

SEQ ID NO: 131 - DNA, 56 bp, synthetic construct
  misc_feature 1..56: note = SORT1_3_F
  source 1..56: mol_type = other DNA
ggctaccgtctctcagtggcggaggcggctcaggcggaaagaaatacgtgtgcggc

SEQ ID NO: 132 - DNA, 85 bp, synthetic construct
  misc_feature 1..85: note = SORT1_3_R
  source 1..85: mol_type = other DNA
ggctaccgtctctgtagctccgcttccagcgtaatctggaacatcgtatgggtatccggagccgccctcaagcagatcctcgtcg

SEQ ID NO: 133 - DNA, 57 bp, synthetic construct
  misc_feature 1..57: note = SORT1_TM_3_F
  source 1..57: mol_type = other DNA
ggctaccgtctctcagtggcggaggcggctcaggcggaagcgtgccaatcatcctgg

SEQ ID NO: 134 - DNA, 35 bp, synthetic construct
  misc_feature 1..35: note = TrxWT_1_F
  source 1..35: mol_type = other DNA
ggctaccgtctcaccatggtgaagcagatcgagag

SEQ ID NO: 135 - DNA, 55 bp, synthetic construct
  misc_feature 1..55: note = TrxWT_1_R
  source 1..55: mol_type = other DNA
ggctaccgtctcatcctccgccgccagatccgccaactagttcgttgatggtggc

SEQ ID NO: 136 - DNA, 58 bp, synthetic construct
  misc_feature 1..58: note = TrxWT_3_F
  source 1..58: mol_type = other DNA
ggctaccgtctctcagtggcggaggcggctcaggcggagtcaagcagatcgagagcaa

SEQ ID NO: 137 - DNA, 87 bp, synthetic construct
  misc_feature 1..87: note = TrxWT_3_R
  source 1..87: mol_type = other DNA
ggctaccgtctctgtagctccgcttccagcgtaatctggaacatcgtatgggtatccggagccgccaactagttcgttgatggtggc

SEQ ID NO: 138 - DNA, 53 bp, synthetic construct; identical to SEQ ID NO: 130
  misc_feature 1..53: note = TrxWT_SORT1_1_R
  source 1..53: mol_type = other DNA

SEQ ID NO: 139 - DNA, 37 bp, synthetic construct
  misc_feature 1..37: note = Ubi_1_F
  source 1..37: mol_type = other DNA
ggctaccgtctcaccatgcagatcttcgtgaaaaccc

SEQ ID NO: 140 - DNA, 55 bp, synthetic construct
  misc_feature 1..55: note = Ubi_1_R
  source 1..55: mol_type = other DNA
ggctaccgtctcatcctccgccgccagatccgcctcttccacctctcagtctcag

SEQ ID NO: 141 - DNA, 60 bp, synthetic construct
  misc_feature 1..60: note = Ubi_3_F
  source 1..60: mol_type = other DNA
ggctaccgtctctcagtggcggaggcggctcaggcggacagatcttcgtgaaaaccctga

SEQ ID NO: 142 - DNA, 85 bp, synthetic construct
  misc_feature 1..85: note = Ubi_3_R
  source 1..85: mol_type = other DNA
ggctaccgtctctgtagctccgcttccagcgtaatctggaacatcgtatgggtatccggagccgcctccacctctcagtctcagc

SEQ ID NO: 143 - DNA, 34 bp, synthetic construct
  misc_feature 1..34: note = NcoI_Epitope_F
  source 1..34: mol_type = other DNA
ccaaggccaccatggagttcaagcacatcaaggc

SEQ ID NO: 144 - DNA, 31 bp, synthetic construct
  misc_feature 1..31: note = XhoI_EGFP_R
  source 1..31: mol_type = other DNA
ctgtattctcgagtttacttgtacagctcgt

SEQ ID NO: 145 - protein, 105 aa, synthetic construct
  REGION 1..105: note = TRXmt_PRT
MVKQIESKTAFQEALDAAGDKLVVVDFSATWSGPSKMIKPFFHSLSEKYSNVIFLEVDVDDSQDVASESEVKSMPTFQFFKKGQKVGEFSGANKEKLEATINELV

SEQ ID NO: 146 - DNA, 315 bp, synthetic construct
  misc_feature 1..315: note = TRXmt_gene
  source 1..315: mol_type = other DNA
atggtgaagcagatcgagagcaagaccgccttccaagaggcccttgatgccgctggcgataagctggtggtggtggatttttccgccacttggagcggccccagcaagatgatcaagccattcttccacagcctgagcgagaagtacagcaacgtgatcttcctggaagtggacgtggacgacagccaggatgtggcctctgagagcgaagtgaagtccatgcctaccttccagttcttcaagaagggccagaaagtcggcgagttcagcggcgccaacaaagagaagctggaagccaccatcaacgagctggtg

SEQ ID NO: 147 - protein, 9 aa, synthetic construct
  REGION 1..9: note = NY-ESO-1
SLLMWITQC

SEQ ID NO: 148 - protein, 9 aa, synthetic construct
  REGION 1..9: note = MAGE-A3
FLWGPRALV

SEQ ID NO: 149 - protein, 9 aa, synthetic construct
  REGION 1..9: note = Survivin
LMLGEFLKL

SEQ ID NO: 150 - protein, 9 aa, synthetic construct
  REGION 1..9: note = Multi MAGE-A
YLEYRQVPV

SEQ ID NO: 151 - protein, 10 aa, synthetic construct
  REGION 1..10: note = Melan A
ELAGIGILTV